European Patent Specification EP 3 680 334 B1, published March 25, 2026. Title: Double-stranded RNA Molecule Targeting CKIP-1 and Use Thereof. Applicant: BEIJING TIDE PHARMACEUTICAL CO., LTD. The sequence listing filed with the application follows.

SEQUENCE LISTING (192 sequences)

SEQ ID NO: 1 - RNA, 19 nt, Artificial Sequence
  si-TD037 sense
aaggucggcuggguccgga

SEQ ID NO: 2 - RNA, 19 nt, Artificial Sequence
  si-TD037 antisense
uccggacccagccgaccuu

SEQ ID NO: 3 - RNA, 19 nt, Artificial Sequence
  si-TD040 sense
gucggcuggguccggaaau

SEQ ID NO: 4 - RNA, 19 nt, Artificial Sequence
  si-TD040 antisense
auuuccggacccagccgac

SEQ ID NO: 5 - RNA, 19 nt, Artificial Sequence
  si-TD042 sense
cggcuggguccggaaauuc

SEQ ID NO: 6 - RNA, 19 nt, Artificial Sequence
  si-TD042 antisense
gaauuuccggacccagccg

SEQ ID NO: 7 - RNA, 19 nt, Artificial Sequence
  si-TD044 sense
gcuggguccggaaauucug

SEQ ID NO: 8 - RNA, 19 nt, Artificial Sequence
  si-TD044 antisense
cagaauuuccggacccagc

SEQ ID NO: 9 - RNA, 19 nt, Artificial Sequence
  si-TD050 sense
uccggaaauucugcgggaa

SEQ ID NO: 10 - RNA, 19 nt, Artificial Sequence
  si-TD050 antisense
uucccgcagaauuuccgga

SEQ ID NO: 11 - RNA, 19 nt, Artificial Sequence
  si-TD057 sense
auucugcgggaaagggauu

SEQ ID NO: 12 - RNA, 19 nt, Artificial Sequence
  si-TD057 antisense
aaucccuuucccgcagaau

SEQ ID NO: 13 - RNA, 19 nt, Artificial Sequence
  si-TD058 sense
uucugcgggaaagggauuu

SEQ ID NO: 14 - RNA, 19 nt, Artificial Sequence
  si-TD058 antisense
aaaucccuuucccgcagaa

SEQ ID NO: 15 - RNA, 19 nt, Artificial Sequence
  si-TD060 sense
cugcgggaaagggauuuuc

SEQ ID NO: 16 - RNA, 19 nt, Artificial Sequence
  si-TD060 antisense
gaaaaucccuuucccgcag

SEQ ID NO: 17 - RNA, 19 nt, Artificial Sequence
  si-TD061 sense
ugcgggaaagggauuuuca

SEQ ID NO: 18 - RNA, 19 nt, Artificial Sequence
  si-TD061 antisense
ugaaaaucccuuucccgca

SEQ ID NO: 19 - RNA, 19 nt, Artificial Sequence
  si-TD062 sense
gcgggaaagggauuuucag

SEQ ID NO: 20 - RNA, 19 nt, Artificial Sequence
  si-TD062 antisense
cugaaaaucccuuucccgc

SEQ ID NO: 21 - RNA, 19 nt, Artificial Sequence
  si-TD064 sense
gggaaagggauuuucaggg

SEQ ID NO: 22 - RNA, 19 nt, Artificial Sequence
  si-TD064 antisense
cccugaaaaucccuuuccc

SEQ ID NO: 23 - RNA, 19 nt, Artificial Sequence
  si-TD065 sense
ggaaagggauuuucaggga

SEQ ID NO: 24 - RNA, 19 nt, Artificial Sequence
  si-TD065 antisense
ucccugaaaaucccuuucc

SEQ ID NO: 25 - RNA, 19 nt, Artificial Sequence
  si-TD066 sense
gaaagggauuuucagggag

SEQ ID NO: 26 - RNA, 19 nt, Artificial Sequence
  si-TD066 antisense
cucccugaaaaucccuuuc

SEQ ID NO: 27 - RNA, 19 nt, Artificial Sequence
  si-TD067 sense
aaagggauuuucagggaga

SEQ ID NO: 28 - RNA, 19 nt, Artificial Sequence
  si-TD067 antisense
ucucccugaaaaucccuuu

SEQ ID NO: 29 - RNA, 19 nt, Artificial Sequence
  si-TD068 sense
aagggauuuucagggagau

SEQ ID NO: 30 - RNA, 19 nt, Artificial Sequence
  si-TD068 antisense
aucucccugaaaaucccuu

SEQ ID NO: 31 - RNA, 19 nt, Artificial Sequence
  si-TD070 sense
gggauuuucagggagauuu

SEQ ID NO: 32 - RNA, 19 nt, Artificial Sequence
  si-TD070 antisense
aaaucucccugaaaauccc

SEQ ID NO: 33 - RNA, 19 nt, Artificial Sequence
  si-TD072 sense
gauuuucagggagauuugg

SEQ ID NO: 34 - RNA, 19 nt, Artificial Sequence
  si-TD072 antisense
ccaaaucucccugaaaauc

SEQ ID NO: 35 - RNA, 19 nt, Artificial Sequence
  si-TD074 sense
uuuucagggagauuuggaa

SEQ ID NO: 36 - RNA, 19 nt, Artificial Sequence
  si-TD074 antisense
uuccaaaucucccugaaaa

SEQ ID NO: 37 - RNA, 19 nt, Artificial Sequence
  si-TD076 sense
uucagggagauuuggaaaa

SEQ ID NO: 38 - RNA, 19 nt, Artificial Sequence
  si-TD076 antisense
uuuuccaaaucucccugaa

SEQ ID NO: 39 - RNA, 19 nt, Artificial Sequence
  si-TD078 sense
cagggagauuuggaaaaac

SEQ ID NO: 40 - RNA, 19 nt, Artificial Sequence
  si-TD078 antisense
guuuuuccaaaucucccug

SEQ ID NO: 41 - RNA, 19 nt, Artificial Sequence
  si-TD080 sense
gggagauuuggaaaaaccg

SEQ ID NO: 42 - RNA, 19 nt, Artificial Sequence
  si-TD080 antisense
cgguuuuuccaaaucuccc

SEQ ID NO: 43 - RNA, 19 nt, Artificial Sequence
  si-TD082 sense
gagauuuggaaaaaccgcu

SEQ ID NO: 44 - RNA, 19 nt, Artificial Sequence
  si-TD082 antisense
agcgguuuuuccaaaucuc

SEQ ID NO: 45 - RNA, 19 nt, Artificial Sequence
  si-TD084 sense
gauuuggaaaaaccgcuau

SEQ ID NO: 46 - RNA, 19 nt, Artificial Sequence
  si-TD084 antisense
auagcgguuuuuccaaauc

SEQ ID NO: 47 - RNA, 19 nt, Artificial Sequence
  si-TD087 sense
uuggaaaaaccgcuaugug

SEQ ID NO: 48 - RNA, 19 nt, Artificial Sequence
  si-TD087 antisense
cacauagcgguuuuuccaa

SEQ ID NO: 49 - RNA, 19 nt, Artificial Sequence
  si-TD089 sense
ggaaaaaccgcuauguggu

SEQ ID NO: 50 - RNA, 19 nt, Artificial Sequence
  si-TD089 antisense
accacauagcgguuuuucc

SEQ ID NO: 51 - RNA, 19 nt, Artificial Sequence
  si-TD093 sense
aaaccgcuauguggugcug

SEQ ID NO: 52 - RNA, 19 nt, Artificial Sequence
  si-TD093 antisense
cagcaccacauagcgguuu

SEQ ID NO: 53 - RNA, 19 nt, Artificial Sequence
  si-TD094 sense
aaccgcuauguggugcuga

SEQ ID NO: 54 - RNA, 19 nt, Artificial Sequence
  si-TD094 antisense
ucagcaccacauagcgguu

SEQ ID NO: 55 - RNA, 19 nt, Artificial Sequence
  si-TD096 sense
ccgcuauguggugcugaaa

SEQ ID NO: 56 - RNA, 19 nt, Artificial Sequence
  si-TD096 antisense
uuucagcaccacauagcgg

SEQ ID NO: 57 - RNA, 19 nt, Artificial Sequence
  si-TD097 sense
cgcuauguggugcugaaag

SEQ ID NO: 58 - RNA, 19 nt, Artificial Sequence
  si-TD097 antisense
cuuucagcaccacauagcg

SEQ ID NO: 59 - RNA, 19 nt, Artificial Sequence
  si-TD098 sense
gcuauguggugcugaaagg

SEQ ID NO: 60 - RNA, 19 nt, Artificial Sequence
  si-TD098 antisense
ccuuucagcaccacauagc

SEQ ID NO: 61 - RNA, 19 nt, Artificial Sequence
  si-TD136 sense
gagaaggagguaaaagaug

SEQ ID NO: 62 - RNA, 19 nt, Artificial Sequence
  si-TD136 antisense
caucuuuuaccuccuucuc

SEQ ID NO: 63 - RNA, 19 nt, Artificial Sequence
  si-TD137 sense
agaaggagguaaaagauga

SEQ ID NO: 64 - RNA, 19 nt, Artificial Sequence
  si-TD137 antisense
ucaucuuuuaccuccuucu

SEQ ID NO: 65 - RNA, 19 nt, Artificial Sequence
  si-TD138 sense
gaaggagguaaaagaugag

SEQ ID NO: 66 - RNA, 19 nt, Artificial Sequence
  si-TD138 antisense
cucaucuuuuaccuccuuc

SEQ ID NO: 67 - RNA, 19 nt, Artificial Sequence
  si-TD139 sense
aaggagguaaaagaugaga

SEQ ID NO: 68 - RNA, 19 nt, Artificial Sequence
  si-TD139 antisense
ucucaucuuuuaccuccuu

SEQ ID NO: 69 - RNA, 19 nt, Artificial Sequence
  si-TD140 sense
aggagguaaaagaugagaa

SEQ ID NO: 70 - RNA, 19 nt, Artificial Sequence
  si-TD140 antisense
uucucaucuuuuaccuccu

SEQ ID NO: 71 - RNA, 19 nt, Artificial Sequence
  si-TD141 sense
ggagguaaaagaugagaaa

SEQ ID NO: 72 - RNA, 19 nt, Artificial Sequence
  si-TD141 antisense
uuucucaucuuuuaccucc

SEQ ID NO: 73 - RNA, 19 nt, Artificial Sequence
  si-TD143 sense
agguaaaagaugagaaaaa

SEQ ID NO: 74 - RNA, 19 nt, Artificial Sequence
  si-TD143 antisense
uuuuucucaucuuuuaccu

SEQ ID NO: 75 - RNA, 19 nt, Artificial Sequence
  si-TD181 sense
cugagugacuaugagaagu

SEQ ID NO: 76 - RNA, 19 nt, Artificial Sequence
  si-TD181 antisense
acuucucauagucacucag

SEQ ID NO: 77 - RNA, 19 nt, Artificial Sequence
  si-TD179 sense
accugagugacuaugagaa

SEQ ID NO: 78 - RNA, 19 nt, Artificial Sequence
  si-TD179 antisense
uucucauagucacucaggu

SEQ ID NO: 79 - RNA, 19 nt, Artificial Sequence
  si-TD178 sense
gaccugagugacuaugaga

SEQ ID NO: 80 - RNA, 19 nt, Artificial Sequence
  si-TD178 antisense
ucucauagucacucagguc

SEQ ID NO: 81 - RNA, 19 nt, Artificial Sequence
  si-TD177 sense
ugaccugagugacuaugag

SEQ ID NO: 82 - RNA, 19 nt, Artificial Sequence
  si-TD177 antisense
cucauagucacucagguca

SEQ ID NO: 83 - RNA, 19 nt, Artificial Sequence
  si-TD176 sense
uugaccugagugacuauga

SEQ ID NO: 84 - RNA, 19 nt, Artificial Sequence
  si-TD176 antisense
ucauagucacucaggucaa

SEQ ID NO: 85 - RNA, 19 nt, Artificial Sequence
  si-TD224 sense
gcaggagcaagaaaaauca

SEQ ID NO: 86 - RNA, 19 nt, Artificial Sequence
  si-TD224 antisense
ugauuuuucuugcuccugc

SEQ ID NO: 87 - RNA, 19 nt, Artificial Sequence
  si-TD221 sense
agagcaggagcaagaaaaa

SEQ ID NO: 88 - RNA, 19 nt, Artificial Sequence
  si-TD221 antisense
uuuuucuugcuccugcucu

SEQ ID NO: 89 - RNA, 19 nt, Artificial Sequence
  si-TD217 sense
uccaagagcaggagcaaga

SEQ ID NO: 90 - RNA, 19 nt, Artificial Sequence
  si-TD217 antisense
ucuugcuccugcucuugga

SEQ ID NO: 91 - RNA, 19 nt, Artificial Sequence
  si-TD380 sense
ugaggaggacagcuaucuu

SEQ ID NO: 92 - RNA, 19 nt, Artificial Sequence
  si-TD380 antisense
aagauagcuguccuccuca

SEQ ID NO: 93 - RNA, 19 nt, Artificial Sequence
  si-TD378 sense
guugaggaggacagcuauc

SEQ ID NO: 94 - RNA, 19 nt, Artificial Sequence
  si-TD378 antisense
gauagcuguccuccucaac

SEQ ID NO: 95 - RNA, 19 nt, Artificial Sequence
  si-TD376 sense
ccguugaggaggacagcua

SEQ ID NO: 96 - RNA, 19 nt, Artificial Sequence
  si-TD376 antisense
uagcuguccuccucaacgg

SEQ ID NO: 97 - RNA, 19 nt, Artificial Sequence
  si-TD372 sense
gucaccguugaggaggaca

SEQ ID NO: 98 - RNA, 19 nt, Artificial Sequence
  si-TD372 antisense
uguccuccucaacggugac

SEQ ID NO: 99 - RNA, 19 nt, Artificial Sequence
  si-TD370 sense
aggucaccguugaggagga

SEQ ID NO: 100 - RNA, 19 nt, Artificial Sequence
  si-TD370 antisense
uccuccucaacggugaccu

SEQ ID NO: 101 - RNA, 19 nt, Artificial Sequence
  si-TD364 sense
uggaugaggucaccguuga

SEQ ID NO: 102 - RNA, 19 nt, Artificial Sequence
  si-TD364 antisense
ucaacggugaccucaucca

SEQ ID NO: 103 - RNA, 19 nt, Artificial Sequence
  si-TD362 sense
cuuggaugaggucaccguu

SEQ ID NO: 104 - RNA, 19 nt, Artificial Sequence
  si-TD362 antisense
aacggugaccucauccaag

SEQ ID NO: 105 - RNA, 19 nt, Artificial Sequence
  si-TD358 sense
guaucuuggaugaggucac

SEQ ID NO: 106 - RNA, 19 nt, Artificial Sequence
  si-TD358 antisense
gugaccucauccaagauac

SEQ ID NO: 107 - RNA, 19 nt, Artificial Sequence
  si-TD451 sense
aggaagacccuuccccuga

SEQ ID NO: 108 - RNA, 19 nt, Artificial Sequence
  si-TD451 antisense
ucaggggaagggucuuccu

SEQ ID NO: 109 - RNA, 19 nt, Artificial Sequence
  si-TD443 sense
gauccaagaggaagacccu

SEQ ID NO: 110 - RNA, 19 nt, Artificial Sequence
  si-TD443 antisense
agggucuuccucuuggauc

SEQ ID NO: 111 - RNA, 19 nt, Artificial Sequence
  si-TD509 sense
ggacaagucuguggcccag

SEQ ID NO: 112 - RNA, 19 nt, Artificial Sequence
  si-TD509 antisense
cugggccacagacuugucc

SEQ ID NO: 113 - RNA, 19 nt, Artificial Sequence
  si-TD508 sense
uggacaagucuguggccca

SEQ ID NO: 114 - RNA, 19 nt, Artificial Sequence
  si-TD508 antisense
ugggccacagacuugucca

SEQ ID NO: 115 - RNA, 19 nt, Artificial Sequence
  si-TD577 sense
gccucccuggaggagaucc

SEQ ID NO: 116 - RNA, 19 nt, Artificial Sequence
  si-TD577 antisense
ggaucuccuccagggaggc

SEQ ID NO: 117 - RNA, 19 nt, Artificial Sequence
  si-TD611 sense
gguagcaaggaaacuggag

SEQ ID NO: 118 - RNA, 19 nt, Artificial Sequence
  si-TD611 antisense
cuccaguuuccuugcuacc

SEQ ID NO: 119 - RNA, 19 nt, Artificial Sequence
  si-TD609 sense
cugguagcaaggaaacugg

SEQ ID NO: 120 - RNA, 19 nt, Artificial Sequence
  si-TD609 antisense
ccaguuuccuugcuaccag

SEQ ID NO: 121 - RNA, 19 nt, Artificial Sequence
  si-TD607 sense
accugguagcaaggaaacu

SEQ ID NO: 122 - RNA, 19 nt, Artificial Sequence
  si-TD607 antisense
aguuuccuugcuaccaggu

SEQ ID NO: 123 - RNA, 19 nt, Artificial Sequence
  si-TD604 sense
aggaccugguagcaaggaa

SEQ ID NO: 124 - RNA, 19 nt, Artificial Sequence
  si-TD604 antisense
uuccuugcuaccagguccu

SEQ ID NO: 125 - RNA, 19 nt, Artificial Sequence
  si-TD600 sense
auccaggaccugguagcaa

SEQ ID NO: 126 - RNA, 19 nt, Artificial Sequence
  si-TD600 antisense
uugcuaccagguccuggau

SEQ ID NO: 127 - RNA, 19 nt, Artificial Sequence
  si-TD598 sense
ggauccaggaccugguagc

SEQ ID NO: 128 - RNA, 19 nt, Artificial Sequence
  si-TD598 antisense
gcuaccagguccuggaucc

SEQ ID NO: 129 - RNA, 19 nt, Artificial Sequence
  si-TD596 sense
ccggauccaggaccuggua

SEQ ID NO: 130 - RNA, 19 nt, Artificial Sequence
  si-TD596 antisense
uaccagguccuggauccgg

SEQ ID NO: 131 - RNA, 19 nt, Artificial Sequence
  si-TD588 sense
cagcugucccggauccagg

SEQ ID NO: 132 - RNA, 19 nt, Artificial Sequence
  si-TD588 antisense
ccuggauccgggacagcug

SEQ ID NO: 133 - RNA, 19 nt, Artificial Sequence
  si-TD587 sense
gcagcugucccggauccag

SEQ ID NO: 134 - RNA, 19 nt, Artificial Sequence
  si-TD587 antisense
cuggauccgggacagcugc

SEQ ID NO: 135 - RNA, 19 nt, Artificial Sequence
  si-TD585 sense
gggcagcugucccggaucc

SEQ ID NO: 136 - RNA, 19 nt, Artificial Sequence
  si-TD585 antisense
ggauccgggacagcugccc

SEQ ID NO: 137 - RNA, 19 nt, Artificial Sequence
  si-TD720 sense
gagcugagagaccuguaca

SEQ ID NO: 138 - RNA, 19 nt, Artificial Sequence
  si-TD720 antisense
uguacaggucucucagcuc

SEQ ID NO: 139 - RNA, 19 nt, Artificial Sequence
  si-TD718 sense
gggagcugagagaccugua

SEQ ID NO: 140 - RNA, 19 nt, Artificial Sequence
  si-TD718 antisense
uacaggucucucagcuccc

SEQ ID NO: 141 - RNA, 19 nt, Artificial Sequence
  si-TD743 sense
gacucccaccucagacaga

SEQ ID NO: 142 - RNA, 19 nt, Artificial Sequence
  si-TD743 antisense
ucugucugaggugggaguc

SEQ ID NO: 143 - RNA, 19 nt, Artificial Sequence
  si-TD145 sense
guaaaagaugagaaaaaua

SEQ ID NO: 144 - RNA, 19 nt, Artificial Sequence
  si-TD145 antisense
uauuuuucucaucuuuuac

SEQ ID NO: 145 - RNA, 19 nt, Artificial Sequence
  si-TD480 sense
ucuugugcugagagcuuuc

SEQ ID NO: 146 - RNA, 19 nt, Artificial Sequence
  si-TD480 antisense
gaaagcucucagcacaaga

SEQ ID NO: 147 - RNA, 19 nt, Artificial Sequence
  si-TD483 sense
ugugcugagagcuuucggg

SEQ ID NO: 148 - RNA, 19 nt, Artificial Sequence
  si-TD483 antisense
cccgaaagcucucagcaca

SEQ ID NO: 149 - RNA, 19 nt, Artificial Sequence
  si-TD736 sense
acagacagauggaccugca

SEQ ID NO: 150 - RNA, 19 nt, Artificial Sequence
  si-TD736 antisense
ugcagguccaucugucugu

SEQ ID NO: 151 - RNA, 19 nt, Artificial Sequence
  si-TD734 sense
guacagacagauggaccug

SEQ ID NO: 152 - RNA, 19 nt, Artificial Sequence
  si-TD734 antisense
cagguccaucugucuguac

SEQ ID NO: 153 - RNA, 19 nt, Artificial Sequence
  si-TD730 sense
accuguacagacagaugga

SEQ ID NO: 154 - RNA, 19 nt, Artificial Sequence
  si-TD730 antisense
uccaucugucuguacaggu

SEQ ID NO: 155 - RNA, 19 nt, Artificial Sequence
  si-TD726 sense
agagaccuguacagacaga

SEQ ID NO: 156 - RNA, 19 nt, Artificial Sequence
  si-TD726 antisense
ucugucuguacaggucucu

SEQ ID NO: 157 - RNA, 19 nt, Artificial Sequence
  si-TD723 sense
cugagagaccuguacagac

SEQ ID NO: 158 - RNA, 19 nt, Artificial Sequence
  si-TD723 antisense
gucuguacaggucucucag

SEQ ID NO: 159 - RNA, 19 nt, Artificial Sequence
  si-TD717 sense
agggagcugagagaccugu

SEQ ID NO: 160 - RNA, 19 nt, Artificial Sequence
  si-TD717 antisense
acaggucucucagcucccu

SEQ ID NO: 161 - RNA, 19 nt, Artificial Sequence
  si-7 sense
ugggagaugggaagcgaaa

SEQ ID NO: 162 - RNA, 19 nt, Artificial Sequence
  si-7 antisense
uuucgcuucccaucuccca

SEQ ID NO: 163 - RNA, 19 nt, Artificial Sequence
  si-10 sense
cagacaaaggggccaccua

SEQ ID NO: 164 - RNA, 19 nt, Artificial Sequence
  si-10 antisense
uagguggccccuuugucug

SEQ ID NO: 165 - RNA, 19 nt, Artificial Sequence
  si-1 sense
ggaccugguagcaaggaaa

SEQ ID NO: 166 - RNA, 19 nt, Artificial Sequence
  si-1 antisense
uuuccuugcuaccaggucc

SEQ ID NO: 167 - DNA, 20 bp, Artificial Sequence
  hCIKP1-F
ggaaccaacctcttgtgctg

SEQ ID NO: 168 - DNA, 20 bp, Artificial Sequence
  hCIKP1-R
gtcaacttcttgggtgcctg

SEQ ID NO: 169 - DNA, 23 bp, Artificial Sequence
  hGADPH-F
catgagaagtatgacaacagcct

SEQ ID NO: 170 - DNA, 22 bp, Artificial Sequence
  hGADPH-R
agtccttccacgataccaaagt

SEQ ID NO: 171 - DNA, 18 bp, Artificial Sequence
  mouse TNF-a-F
tcagcgaggacagcaagg

SEQ ID NO: 172 - DNA, 22 bp, Artificial Sequence
  mouse TNFa-R
agtgagtgaaagggacagaacc

SEQ ID NO: 173 - DNA, 20 bp, Artificial Sequence
  mouse IL6-F
ccttcttgggactgatgctg

SEQ ID NO: 174 - DNA, 22 bp, Artificial Sequence
  mouse IL6-R
ttgggagtggtatcctctgtga

SEQ ID NO: 175 - DNA, 24 bp, Artificial Sequence
  mouse GAPDH-F
ccttcattgacctcaactacatgg

SEQ ID NO: 176 - DNA, 20 bp, Artificial Sequence
  mouse GAPDH-R
ctcgctcctggaagatggtg

SEQ ID NO: 177 - DNA, 20 bp, Artificial Sequence
  ALP-F
gtcagctccaccacaaccct

SEQ ID NO: 178 - DNA, 20 bp, Artificial Sequence
  ALP-R
gccctcattggccttcaccc

SEQ ID NO: 179 - DNA, 20 bp, Artificial Sequence
  COL1-F
cactggtgatgctggtcctg

SEQ ID NO: 180 - DNA, 19 bp, Artificial Sequence
  COL1-R
cgaggtcacggtcacgaac

SEQ ID NO: 181 - DNA, 20 bp, Artificial Sequence
  OPN-F
gtaccctgatgctacagacg

SEQ ID NO: 182 - DNA, 20 bp, Artificial Sequence
  OPN-R
ttcataactgtccttcccac

SEQ ID NO: 183 - DNA, 20 bp, Artificial Sequence
  BSP-F
ggcacctcgaagacaacaac

SEQ ID NO: 184 - DNA, 20 bp, Artificial Sequence
  BSP-R
gcccgtgtattcgtactccc

SEQ ID NO: 185 - DNA, 20 bp, Artificial Sequence
  OC-F
agggcagcgaggtagtgaag

SEQ ID NO: 186 - DNA, 20 bp, Artificial Sequence
  OC-R
tgtggtcagccaactcgtca

SEQ ID NO: 187 - DNA, 21 bp, Artificial Sequence
  GAPDH-F
ggcatggactgtggtcatgag

SEQ ID NO: 188 - DNA, 20 bp, Artificial Sequence
  GAPDH-R
tgcaccaccaactgcttagc

SEQ ID NO: 189 - DNA, 19 bp, Artificial Sequence
  mouse IL-17A-F
ctccaccgcaatgaagacc

SEQ ID NO: 190 - DNA, 20 bp, Artificial Sequence
  mouse IL-17A-R
ccctcttcaggaccaggatc

SEQ ID NO: 191 - DNA, 21 bp, Artificial Sequence
  mouse CKIP-1-F
tttctcggccttgggaaaaac

SEQ ID NO: 192 - DNA, 19 bp, Artificial Sequence
  mouse CKIP-1-R
gaggcacatcggctcttct